European Patent Application EP 4 667 571 A1, published December 24, 2025. Title: Artificial MiRNA Construct. Applicant: National University Corporation Tokyo Medical and Dental University. The sequence listing filed with the application follows.

SEQUENCE LISTING (11 sequences)

SEQ ID NO: 1 - RNA, 120 nt, Homo sapiens
  source 1..120: mol_type = transcribed RNA
tctgtcattcgctcccacattctgatgagcaaccgcttccctatttatttatttatttgtttgtttgttttattcattggtctaatttattcaaagggggcaagaagtagcagtgtctgt

SEQ ID NO: 2 - RNA, 120 nt, Homo sapiens
  source 1..120: mol_type = transcribed RNA
aagcaatggttgatgatacttcccacaccacaaatgggacacatggtctgtcaatgagagcataatttaaaaatatatttataaggaaattttacaagggcataaagtaaatacatgcat

SEQ ID NO: 3 - RNA, 11 nt, Homo sapiens
  source 1..11: mol_type = other RNA
tgtttgtttgt

SEQ ID NO: 4 - RNA, 22 nt, synthetic construct
  source 1..22: mol_type = other RNA
ataaataagcctccgggatcca

SEQ ID NO: 5 - RNA, 22 nt, synthetic construct
  source 1..22: mol_type = other RNA
ataaatatgcctccgggatcca

SEQ ID NO: 6 - RNA, 22 nt, synthetic construct
  source 1..22: mol_type = other RNA
aaataaatgcctccgggatcca

SEQ ID NO: 7 - RNA, 22 nt, synthetic construct
  source 1..22: mol_type = other RNA
aacacacacgctgggtctttaa

SEQ ID NO: 8 - RNA, 24 nt, synthetic construct
  source 1..24: mol_type = other RNA
taaaattagcctccgggatccatt

SEQ ID NO: 9 - RNA, 24 nt, synthetic construct
  source 1..24: mol_type = other RNA
tataaattgcctccgggatccatt

SEQ ID NO: 10 - RNA, 24 nt, synthetic construct
  source 1..24: mol_type = other RNA
tggatcccggaggcatatttattt

SEQ ID NO: 11 - RNA, 24 nt, synthetic construct
  source 1..24: mol_type = other RNA
tnnnnnnngcctccgggatccatt